European Patent Application EP 4 552 654 A1, published May 14, 2025. Title: 抗体药物偶联物及其制备方法和用途. Applicant: 苏州宜联生物医药有限公司. Application CN. The sequence listing filed with the application follows.

SEQUENCE LISTING (83 sequences)

SEQ ID NO: 1 - protein, 119 aa, synthetic construct
QVQLQQSGPVLVKPGASVKMSCKASGYTFTDYYMNWVKQSHGKSLEWIGVINPYNGGTNYSQKFKGKATLTVDKSSSTAYMELNSLTSEDSAVYYCARDSNYVGLLDYWGQGTSVTVSS

SEQ ID NO: 2 - protein, 113 aa, synthetic construct
QVQLVESGAEVKKPGSSVKVSCKASGYAFSSHWVNWVRQAPGQGLEWMGQIYPGNGDTNYAQKFQGRVTLTADKSTSTAYMELSSLTSEDTAVYFCARWFAYWGQGTLVTVSS

SEQ ID NO: 3 - protein, 113 aa, synthetic construct
DIVMTQSPSSLAMSVGQRVTINCKSSQSLLDGGNQKNYLAWYQQKVGQPPKLLVYFASIRESGVPDRFIGSGSGTDFTLTISSVQTEDLADYFCQQHYNTPWTFGGGTKLEIK

SEQ ID NO: 4 - protein, 113 aa, synthetic construct
DIQMTQSPSSLSASVGDRVTITCKSSQSLLDGGNQKNYLAWYQQKPGKPPKLLVYFASIRESGVPSRFSGSGSGTDFTLTISSLQPEDFATYYCQQHYNTPWTFGQGTKVEIK

SEQ ID NO: 5 - protein, 119 aa, synthetic construct
EVQLQQSGPVLVKPGASVKMSCKASGYTFTDYYMNWVKQSHGKSLEWIGVINPYNGGTNYSQKFKGKATLTVDKSSSTAYMELNSLTSEDSAVYYCARDSNYVGLLDYWGQGTSVTVSS

SEQ ID NO: 6 - protein, 119 aa, synthetic construct
EVQLVQSGAEVKKPGASVKVSCKASGYTFTDYYMNWVRQAPGQRLEWMGVINPYNGGTNYSQKFQGRVTLTVDKSASTAYMELSSLRSEDTAVYYCARDSNYVGLLDYWGQGTLVTVSS

SEQ ID NO: 7 - protein, 119 aa, synthetic construct
EVQLVQSGAEVKKPGASVKVSCKASGYTFTDYYMNWVRQAPGQRLEWMGVINPYNGGTNYAQKFQGRVTLTVDKSASTAYMELSSLRSEDTAVYYCARDSNYVGLLDYWGQGTLVTVSS

SEQ ID NO: 8 - protein, 107 aa, synthetic construct
DIVLTQSPATLSVTPGDSVSLSCRASQSISNNLHWYQQKSHESPRLLIKYASQSISGIPSRFSGSGSGPDFTLSIDSVETEDFGVYFCQQSNSWPYTFGGGTKLEIK

SEQ ID NO: 9 - protein, 107 aa, synthetic construct
DIVLTQSPATLSLSPGERATLSCRASQSISNNLHWYQQKPGQAPRLLIKYASQSISGIPARFSGSGSGPDFTLTISSLEPEDFAVYFCQQSNSWPYTFGQGTKVEIK

SEQ ID NO: 10 - protein, 125 aa, synthetic construct
EVKLEESGGGLVQPGGSMKLSCAASGFTFSDAWMDWVRQSPEKGLEWIAEIRNKANNHATYYTESVKGRFTISRDDSKSSVYLQMISLRPEDTGIYYCTRNNYGSTWTYYAMDYWGQGTSVTVSS

SEQ ID NO: 11 - protein, 125 aa, synthetic construct
EVQLVESGGGLVQPGGSLRLSCAASGFTFSDAWMDWVRQAPGKGLEWVAEIRNKANNHATYYVDSVKGRFTISRDDAKNSVYLQMNSLRAEDTAVYYCTRNNYGSTWTYYAMDYWGQGTLVTVSS

SEQ ID NO: 12 - protein, 107 aa, synthetic construct
DIQMTQTSSSLSASLGDRVTINCRASQDISNYLNWYQQKPDGTVKLLIYYTSRLHSGVPSRFSGSGSGTDYSLTISNLEHEDIATYFCQQGYTLPLTFGAGTNLELK

SEQ ID NO: 13 - protein, 107 aa, synthetic construct
DIQMTQSPSSLSASVGDRVTITCRASQDISNYLNWYQQKPGKAVKLLIYYTSRLHSGVPSRFSGSGSGTDYTLTISSLQPEDFATYYCQQGYTLPLTFGQGTKVEIK

SEQ ID NO: 14 - protein, 119 aa, synthetic construct
DVQLQESGPGLVKPSQSLSLTCSVTGYSITSDFYWNWIRQFPGNKLEWMGYITYDGSTNYDPSLKNRISITRDTSKNQFFLKLNSVTAEDTATYYCVYGDFNRHAMDYWGQGTSVTVSS

SEQ ID NO: 15 - protein, 119 aa, synthetic construct
QVQLQESGPGLVKPSETLSLTCTVSGYSITSDFYWNWIRQPPGKGLEWIGYITYDGSTNYNPSLKSRVTISRDTSKNQFSLKLSSVTAADTAVYYCVYGDFNRHAMDYWGQGTLVTVSS

SEQ ID NO: 16 - protein, 111 aa, synthetic construct
DIVMSQSPSSLAVSAGEKVTMSCRSSQSLFNSRTRKNYLAWYQQKPGQPPKVLIYWASTRESGVPDRFTGSGSGTDFTLTISSVQAEDLAVYYCEQSFYLFTFGTGTKLEI

SEQ ID NO: 17 - protein, 112 aa, synthetic construct
DIVMTQSPDSLAVSLGERATINCRSSQSLFNSRTRKNYLAWYQQKPGQPPKVLIYWASTRESGVPDRFSGSGSGTDFTLTISSLQAEDVAVYYCEQSFYLFTFGQGTKVEIK

SEQ ID NO: 18 - protein, 120 aa, synthetic construct
EVHLQQSGPVLVKPGPSVKISCKASGFTFTDYYMHWVKQSHGKSLEWIGLVYPYNGDISYNQKFKGKATLTVDTSSSTAYMELNSLTSEDSAVYYCARQGNYVNNAIDYWGQGTSVTVSS

SEQ ID NO: 19 - protein, 120 aa, synthetic construct
EVQLVQSGAEVKKPGASVKVSCKASGFTFTDYYMHWVRQAPGQSLEWMGLVYPYNGDISYAQKFQGRVTLTVDTSISTAYMELSRLRSDDTAVYYCARQGNYVNNAIDYWGQGTLVTVSS

SEQ ID NO: 20 - protein, 120 aa, synthetic construct
EVQLVQSGAEVKKPGASVKVSCKASGFTFTDYYMHWVRQAPGQSLEWMGLVYPYSGDISYAQKFQGRVTLTVDTSISTAYMELSRLRSDDTAVYYCARQGNYVNNAIDYWGQGTLVTVSS

SEQ ID NO: 21 - protein, 106 aa, synthetic construct
DIVMTQSQKFMSTSVGDRVSISCKASQNVGNIIAWYQQKPGQSPKALIYLASYRYSGVPDRFTGSGSGTDFTLTINNVQSEDLAEYFCQQYSDSPYTFGSGTKLEI

SEQ ID NO: 22 - protein, 107 aa, synthetic construct
DIQMTQSPSSLSASVGDRVTITCKASQNVGNIIAWYQQKPGKSPKALIYLASYRYSGVPSRFSGSGSGTDFTLTISSLQPEDVATYFCQQYSDSPYTFGQGTKVEIK

SEQ ID NO: 23 - protein, 5 aa, synthetic construct
SHWVN

SEQ ID NO: 24 - protein, 17 aa, synthetic construct
QIYPGNGDTNYAQKFQG

SEQ ID NO: 25 - protein, 4 aa, synthetic construct
WFAY

SEQ ID NO: 26 - protein, 17 aa, synthetic construct
KSSQSLLDGGNQKNYLA

SEQ ID NO: 27 - protein, 7 aa, synthetic construct
FASIRES

SEQ ID NO: 28 - protein, 9 aa, synthetic construct
QQHYNTPWT

SEQ ID NO: 29 - protein, 8 aa, synthetic construct
GYAFSSHW

SEQ ID NO: 30 - protein, 8 aa, synthetic construct
IYPGNGDT

SEQ ID NO: 31 - protein, 6 aa, synthetic construct
ARWFAY

SEQ ID NO: 32 - protein, 12 aa, synthetic construct
QSLLDGGNQKNY

SEQ ID NO: 33 - protein, 449 aa, synthetic construct
EVQLVQSGAEVKKPGASVKVSCKASGYTFTDYYMNWVRQAPGQRLEWMGVINPYNGGTNYSQKFQGRVTLTVDKSASTAYMELSSLRSEDTAVYYCARDSNYVGLLDYWGQGTLVTVSSASTKGPSVFPLAPSSKSTSGGTAALGCLVKDYFPEPVTVSWNSGALTSGVHTFPAVLQSSGLYSLSSVVTVPSSSLGTQTYICNVNHKPSNTKVDKKVEPKSCDKTHTCPPCPAPELLGGPSVFLFPPKPKDTLMISRTPEVTCVVVDVSHEDPEVKFNWYVDGVEVHNAKTKPREEQYNSTYRVVSVLTVLHQDWLNGKEYKCKVSNKALPAPIEKTISKAKGQPREPQVYTLPPSRDELTKNQVSLTCLVKGFYPSDIAVEWESNGQPENNYKTTPPVLDSDGSFFLYSKLTVDKSRWQQGNVFSCSVMHEALHNHYTQKSLSLSPGK

SEQ ID NO: 34 - protein, 5 aa, synthetic construct
DYYMN

SEQ ID NO: 35 - protein, 17 aa, synthetic construct
VINPYNGGTNYSQKFQG

SEQ ID NO: 36 - protein, 17 aa, synthetic construct
VINPYNGGTNYAQKFQG

SEQ ID NO: 37 - protein, 10 aa, synthetic construct
DSNYVGLLDY

SEQ ID NO: 38 - protein, 11 aa, synthetic construct
RASQSISNNLH

SEQ ID NO: 39 - protein, 7 aa, synthetic construct
YASQSIS

SEQ ID NO: 40 - protein, 9 aa, synthetic construct
QQSNSWPYT

SEQ ID NO: 41 - protein, 8 aa, synthetic construct
GYTFTDYY

SEQ ID NO: 42 - protein, 8 aa, synthetic construct
INPYNGGT

SEQ ID NO: 43 - protein, 12 aa, synthetic construct
ARDSNYVGLLDY

SEQ ID NO: 44 - protein, 6 aa, synthetic construct
QSISNN

SEQ ID NO: 45 - protein, 449 aa, synthetic construct
EVQLVQSGAEVKKPGASVKVSCKASGYTFTDYYMNWVRQAPGQRLEWMGVINPYNGGTNYAQKFQGRVTLTVDKSASTAYMELSSLRSEDTAVYYCARDSNYVGLLDYWGQGTLVTVSSASTKGPSVFPLAPSSKSTSGGTAALGCLVKDYFPEPVTVSWNSGALTSGVHTFPAVLQSSGLYSLSSVVTVPSSSLGTQTYICNVNHKPSNTKVDKKVEPKSCDKTHTCPPCPAPELLGGPSVFLFPPKPKDTLMISRTPEVTCVVVDVSHEDPEVKFNWYVDGVEVHNAKTKPREEQYNSTYRVVSVLTVLHQDWLNGKEYKCKVSNKALPAPIEKTISKAKGQPREPQVYTLPPSRDELTKNQVSLTCLVKGFYPSDIAVEWESNGQPENNYKTTPPVLDSDGSFFLYSKLTVDKSRWQQGNVFSCSVMHEALHNHYTQKSLSLSPGK

SEQ ID NO: 46 - protein, 5 aa, synthetic construct
DAWMD

SEQ ID NO: 47 - protein, 19 aa, synthetic construct
EIRNKANNHATYYVDSVKG

SEQ ID NO: 48 - protein, 14 aa, synthetic construct
NNYGSTWTYYAMDY

SEQ ID NO: 49 - protein, 11 aa, synthetic construct
RASQDISNYLN

SEQ ID NO: 50 - protein, 7 aa, synthetic construct
YTSRLHS

SEQ ID NO: 51 - protein, 9 aa, synthetic construct
QQGYTLPLT

SEQ ID NO: 52 - protein, 8 aa, synthetic construct
GFTFSDAW

SEQ ID NO: 53 - protein, 10 aa, synthetic construct
IRNKANNHAT

SEQ ID NO: 54 - protein, 16 aa, synthetic construct
TRNNYGSTWTYYAMDY

SEQ ID NO: 55 - protein, 6 aa, synthetic construct
QDISNY

SEQ ID NO: 56 - protein, 214 aa, synthetic construct
DIVLTQSPATLSLSPGERATLSCRASQSISNNLHWYQQKPGQAPRLLIKYASQSISGIPARFSGSGSGPDFTLTISSLEPEDFAVYFCQQSNSWPYTFGQGTKVEIKRTVAAPSVFIFPPSDEQLKSGTASVVCLLNNFYPREAKVQWKVDNALQSGNSQESVTEQDSKDSTYSLSSTLTLSKADYEKHKVYACEVTHQGLSSPVTKSFNRGEC

SEQ ID NO: 57 - protein, 6 aa, synthetic construct
SDFYWN

SEQ ID NO: 58 - protein, 16 aa, synthetic construct
YITYDGSTNYNPSLKS

SEQ ID NO: 59 - protein, 10 aa, synthetic construct
GDFNRHAMDY

SEQ ID NO: 60 - protein, 17 aa, synthetic construct
RSSQSLFNSRTRKNYLA

SEQ ID NO: 61 - protein, 7 aa, synthetic construct
WASTRES

SEQ ID NO: 62 - protein, 8 aa, synthetic construct
EQSFYLFT

SEQ ID NO: 63 - protein, 9 aa, synthetic construct
GYSITSDFY

SEQ ID NO: 64 - protein, 7 aa, synthetic construct
ITYDGST

SEQ ID NO: 65 - protein, 12 aa, synthetic construct
VYGDFNRHAMDY

SEQ ID NO: 66 - protein, 12 aa, synthetic construct
QSLFNSRTRKNY

SEQ ID NO: 67 - protein, 450 aa, synthetic construct
EVQLVQSGAEVKKPGASVKVSCKASGFTFTDYYMHWVRQAPGQSLEWMGLVYPYNGDISYAQKFQGRVTLTVDTSISTAYMELSRLRSDDTAVYYCARQGNYVNNAIDYWGQGTLVTVSSASTKGPSVFPLAPSSKSTSGGTAALGCLVKDYFPEPVTVSWNSGALTSGVHTFPAVLQSSGLYSLSSVVTVPSSSLGTQTYICNVNHKPSNTKVDKKVEPKSCDKTHTCPPCPAPELLGGPSVFLFPPKPKDTLMISRTPEVTCVVVDVSHEDPEVKFNWYVDGVEVHNAKTKPREEQYNSTYRVVSVLTVLHQDWLNGKEYKCKVSNKALPAPIEKTISKAKGQPREPQVYTLPPSRDELTKNQVSLTCLVKGFYPSDIAVEWESNGQPENNYKTTPPVLDSDGSFFLYSKLTVDKSRWQQGNVFSCSVMHEALHNHYTQKSLSLSPGK

SEQ ID NO: 68 - protein, 5 aa, synthetic construct
DYYMH

SEQ ID NO: 69 - protein, 17 aa, synthetic construct
LVYPYNGDISYAQKFQG

SEQ ID NO: 70 - protein, 17 aa, synthetic construct
LVYPYSGDISYAQKFQG

SEQ ID NO: 71 - protein, 11 aa, synthetic construct
QGNYVNNAIDY

SEQ ID NO: 72 - protein, 11 aa, synthetic construct
KASQNVGNIIA

SEQ ID NO: 73 - protein, 7 aa, synthetic construct
LASYRYS

SEQ ID NO: 74 - protein, 9 aa, synthetic construct
QQYSDSPYT

SEQ ID NO: 75 - protein, 8 aa, synthetic construct
GFTFTDYY

SEQ ID NO: 76 - protein, 8 aa, synthetic construct
VYPYNGDI

SEQ ID NO: 77 - protein, 8 aa, synthetic construct
VYPYSGDI

SEQ ID NO: 78 - protein, 13 aa, synthetic construct
ARQGNYVNNAIDY

SEQ ID NO: 79 - protein, 6 aa, synthetic construct
QNVGNI

SEQ ID NO: 80 - protein, 450 aa, synthetic construct
EVQLVQSGAEVKKPGASVKVSCKASGFTFTDYYMHWVRQAPGQSLEWMGLVYPYSGDISYAQKFQGRVTLTVDTSISTAYMELSRLRSDDTAVYYCARQGNYVNNAIDYWGQGTLVTVSSASTKGPSVFPLAPSSKSTSGGTAALGCLVKDYFPEPVTVSWNSGALTSGVHTFPAVLQSSGLYSLSSVVTVPSSSLGTQTYICNVNHKPSNTKVDKKVEPKSCDKTHTCPPCPAPELLGGPSVFLFPPKPKDTLMISRTPEVTCVVVDVSHEDPEVKFNWYVDGVEVHNAKTKPREEQYNSTYRVVSVLTVLHQDWLNGKEYKCKVSNKALPAPIEKTISKAKGQPREPQVYTLPPSRDELTKNQVSLTCLVKGFYPSDIAVEWESNGQPENNYKTTPPVLDSDGSFFLYSKLTVDKSRWQQGNVFSCSVMHEALHNHYTQKSLSLSPGK

SEQ ID NO: 81 - protein, 214 aa, synthetic construct
DIQMTQSPSSLSASVGDRVTITCKASQNVGNIIAWYQQKPGKSPKALIYLASYRYSGVPSRFSGSGSGTDFTLTISSLQPEDVATYFCQQYSDSPYTFGQGTKVEIKRTVAAPSVFIFPPSDEQLKSGTASVVCLLNNFYPREAKVQWKVDNALQSGNSQESVTEQDSKDSTYSLSSTLTLSKADYEKHKVYACEVTHQGLSSPVTKSFNRGEC

SEQ ID NO: 82 - protein, 330 aa, synthetic construct [sequence omitted]

SEQ ID NO: 83 - protein, 107 aa, synthetic construct [sequence omitted]